European Patent Application EP 4 245 851 A1, published September 20, 2023. Title: MUTANT CIS-PRENYLTRANSFERASE (CPT) FAMILY PROTEIN, METHOD FOR PRODUCING POLYISOPRENOID, VECTOR, TRANSGENIC PLANT, METHOD FOR PRODUCING PNEUMATIC TIRE, AND METHOD FOR PRODUCING RUBBER PRODUCT. Applicant: SUMITOMO RUBBER INDUSTRIES, LTD. Application EP. The sequence listing filed with the application follows.

SEQUENCE LISTING (24 sequences)

SEQ ID NO: 1 - protein, 290 aa, Hevea brasiliensis
MELYNGERPSVFRLLGKYMRKGLYSILTQGPIPTHIAFILDGNRRFAKKHKLPEGGGHKAGFLALLNVLTYCYELGVKYATIYAFSIDNFRRKPHEVQYVMDLMLEKIEGMIMEESIINAYDICVRFVGNLKLLSEPVKTAADKIMRATANNSKCVLLIAVCYTSTDEIVHAVEESSELNSNEVCNNQELEEANATGSGTVIQIENMESYSGIKLVDLEKNTYINPYPDVLIRTSGETRLSNYLLWQTTNCILYSPHALWPEIGLRHVVWAVINFQRHYSYLEKHKEYLK

SEQ ID NO: 2 - DNA, 873 bp, Hevea brasiliensis
  source 1..873: mol_type = genomic DNA
atggaattatacaacggtgagaggccaagtgtgttcagacttttagggaagtatatgagaaaagggttatatagcatcctaacccagggtcccatccctactcatattgccttcatattggatggaaacaggaggtttgctaagaagcataaactgccagaaggaggtggtcataaggctggatttttagctcttctgaacgtactaacttattgctatgagttaggagtgaaatatgcgactatctatgcctttagcatcgataattttcgaaggaaacctcatgaggttcagtacgtaatggatctaatgctggagaagattgaagggatgatcatggaagaaagtatcatcaatgcatatgatatttgcgtacgttttgtgggtaacctgaagcttttaagtgagccagtcaagaccgcagcagataagattatgagggctactgccaacaattccaaatgtgtgcttctcattgctgtatgctatacttcaactgatgagatcgtgcatgctgttgaagaatcctctgaattgaactccaatgaagtttgtaacaatcaagaattggaggaggcaaatgcaactggaagcggtactgtgattcaaattgagaacatggagtcgtattctggaataaaacttgtagaccttgagaaaaacacctacataaatccttatcctgatgttctgattcgaacttctggggagacccgtctgagcaactacttactttggcagactactaattgcatactgtattctcctcatgcactgtggccagagattggtcttcgacacgtggtgtgggcagtaattaacttccaacgtcattattcttacttggagaaacataaggaatacttaaaataa

SEQ ID NO: 3 - protein, 302 aa, Arabidopsis thaliana
MLSILSSLLSLLFLFIISCFFITSHFWFPLSLPKILGFIKITSSRDDYDNEQRDEGTYVVGVEELQRELMPRHVAVIMDGNRRWAKRAGLLTSQGHEAGAKRLIEFSELCFKLGIHTVSAFAFSTENWGRHKIEVKCLMSLIQHYLKSKIQYFQREETRVSVIGNLTKIPESLLRTVQEIEEATRSYKKKHLILAIDYSGRLDILRACKSIVKKSEKGLIREEDVDEALIERELLTNCTEFPSPDLLIRTSGEQRISNFFLWQLAYTELFFSPVLWPDFDKDKLLEALVSYQRRERRFGCRV

SEQ ID NO: 4 - protein, 368 aa, Hevea brasiliensis
MEIFEAGRPSVLASLGRFIRKCIFRILSIGPIPSHVAFIMDGNRRFAKKEKLEEGSGHRAGSLALMSTLKYCYELGVKYVTIYAFSIDNFRRRPDEVQLIMDLILEKIEGLLRDENVVNAYGIRVRFVGTLKLLSEPVRVAAEKVARASAKNTKFVLVICIAYSSTDEIVHAVQESCKYKLNKIEPSNSNRACNDANEQVEENGKKIDSTITHGVQESCKDETDKSRTINAKPMYNGVTKEAGGTDNANTVIVNSIGDKWDDAHELEATRTGNGVISVEEIDKMLSHSSIKLVDIEKKLHMAVAPDPDILVRTSGESRLSNFLLWQTSNCSLYSPKALWPEIGLRHLVWAVITFQRNHSYLEKKKKQL

SEQ ID NO: 5 - DNA, 909 bp, Arabidopsis thaliana
  source 1..909: mol_type = genomic DNA
atgttgtctattctctcttctcttttatctctcctttttctgtttatcatctcttgtttcttcatcacaagccatttttggttccctctttccttgccaaaaatactcggattcatcaaaatcacatcttcgagagacgattatgacaacgagcaacgtgacgagggaacttatgtggtaggagtggaggagctacaaagagagctgatgccaagacatgtggcagtgataatggacggaaaccggagatgggccaaacgggccggattgctgacgtcacaaggccacgaggccggagctaaacggcttatagagttctccgagctttgctttaaattggggattcatacagtttcagcttttgccttctccacagagaattggggaagacacaagattgaggttaagtgcttgatgtctttgatccaacattacctcaagtccaagatccaatatttccaaagagaggaaactcgagtttctgttatcgggaacctaacgaagatccctgagtctctcctccgaacagtccaagagatagaggaagctacgagaagctataagaagaagcatctcatattggcaatagattacagcgggagattagacatcttgcgagcttgcaagagtattgtgaagaaatcagaaaaagggttgatccgagaggaagatgtagacgaggcattgatcgaaagagagcttctgacaaattgtactgagttcccaagtcctgatctattgattaggacaagtggagaacagaggattagtaacttcttcttgtggcaacttgcttatacagagctcttcttctcgccggtcctttggcctgatttcgataaggataagcttctagaggccctggtttcgtatcagcgccgggaaagacgatttggctgtcgggtttga

SEQ ID NO: 6 - DNA, 1107 bp, Hevea brasiliensis
  source 1..1107: mol_type = genomic DNA
atggaaatatttgaggctggtaggccaagcgtgcttgcaagtttggggagatttatcagaaaatgcatatttcgcattctatcaataggtcccatcccaagtcatgttgccttcataatggatggaaaccggaggtttgctaagaaggagaaactggaagaaggatctggtcacagggctggatctttagctctaatgtccacgcttaagtactgctatgagttgggagtgaagtatgtgactatatatgccttcagcattgataattttagaaggcgacctgatgaggttcagctcataatggatctaatactggagaagattgaggggctgctcagggacgaaaatgttgtcaatgcatatggcatcagagtacgatttgtaggtaccttgaagcttctaagtgagccagtcagggtcgcagcagaaaaagtcgccagggctagtgccaagaataccaagtttgtgcttgtcatttgtatagcctattcttcaactgatgagattgtgcatgctgttcaagaatcttgtaaatataaattgaacaaaattgagccatctaactccaacagggcttgcaatgatgcgaatgaacaagtagaagaaaatggtaagaagatagatagtaccatcacacatggtgttcaagaatcctgcaaagatgaaacagataaatctcgcacaataaacgcaaagccaatgtataatggtgtgaccaaagaagctggagggactgacaatgctaatactgtgatagtaaattccatcggagacaagtgggatgatgctcacgaactggaggcaactagaactggcaatggtgtgatttcagtagaagaaattgataagatgctgtcacattctagcataaagctggtagacattgagaaaaaattgcacatggctgtagcccctgatcctgatatcttggttcgaacttctggagagagccgtctgagcaacttcctactttggcagactagtaactgttcactgtattctccaaaggcactgtggccggagattggcctacgccacttggtgtgggcagtaataaccttccaacgtaatcattcttatttggagaagaaaaagaagcagttgtaa

SEQ ID NO: 7 - protein, 264 aa, synthetic construct
MELYNGERPSVFRLLGKYMRKGLYSILTQGPIPTHVAVIMDGNRRWAKRAGLLTSQGHEAGAKRLIEFSELCFKLGIHTVSAFAFSTENWGRHKIEVKCLMSLIQHYLKSKIQYFQREETRVSVIGNLTKIPESLLRTVQEIEEATRSYKKKHLILAIDYSGRLDILRACKSIVKKSEKGLIREEDVDEALIERELLTNCTEFPSPDLLIRTSGEQRISNFFLWQLAYTELFFSPVLWPDFDKDKLLEALVSYQRRERRFGCRV

SEQ ID NO: 8 - DNA, 795 bp, synthetic construct
  source 1..795: mol_type = other DNA
atggaattatacaacggtgagaggccaagtgtgttcagacttttagggaagtatatgagaaaagggttatatagcatcctaacccagggtcccatccctactcatgtggcagtgataatggacggaaaccggagatgggccaaacgggccggattgctgacgtcacaaggccacgaggccggagctaaacggcttatagagttctccgagctttgctttaaattggggattcatacagtttcagcttttgccttctccacagagaattggggaagacacaagattgaggttaagtgcttgatgtctttgatccaacattacctcaagtccaagatccaatatttccaaagagaggaaactcgagtttctgttatcgggaacctaacgaagatccctgagtctctcctccgaacagtccaagagatagaggaagctacgagaagctataagaagaagcatctcatattggcaatagattacagcgggagattagacatcttgcgagcttgcaagagtattgtgaagaaatcagaaaaagggttgatccgagaggaagatgtagacgaggcattgatcgaaagagagcttctgacaaattgtactgagttcccaagtcctgatctattgattaggacaagtggagaacagaggattagtaacttcttcttgtggcaacttgcttatacagagctcttcttctcgccggtcctttggcctgatttcgataaggataagcttctagaggccctggtttcgtatcagcgccgggaaagacgatttggctgtcgggtttga

SEQ ID NO: 9 - DNA, 417 bp, Hevea brasiliensis
  source 1..417: mol_type = genomic DNA
atggctgaagacgaagacaaccaacaagggcagggggaggggttaaaatatttgggttttgtgcaagacgcggcaacttatgctgtgactaccttctcaaacgtctatctttttgccaaagacaaatctggtccactgcagcctggtgtcgatatcattgagggtccggtgaagaacgtggctgtacctctctataataggttcagttatattcccaatggagctctcaagtttgtagacagcacggttgttgcatctgtcactattatagatcgctctcttcccccaattgtcaaggacgcatctatccaagttgtttcagcaattcgagctgccccagaagctgctcgttctctggcttcttctttgcctgggcagaccaagatacttgctaaggtgttttatggagagaattga

SEQ ID NO: 10 - protein, 138 aa, Hevea brasiliensis
MAEDEDNQQGQGEGLKYLGFVQDAATYAVTTFSNVYLFAKDKSGPLQPGVDIIEGPVKNVAVPLYNRFSYIPNGALKFVDSTVVASVTIIDRSLPPIVKDASIQVVSAIRAAPEAARSLASSLPGQTKILAKVFYGEN

SEQ ID NO: 11 - DNA, 34 bp, synthetic construct
  misc_feature 1..34: note = PRIMER-1
  source 1..34: mol_type = other DNA
tttggatccgatggaattatacaacggtgagagg

SEQ ID NO: 12 - DNA, 39 bp, synthetic construct
  misc_feature 1..39: note = PRIMER-2
  source 1..39: mol_type = other DNA
tttgcggccgcttattttaagtattccttatgtttctcc

SEQ ID NO: 13 - DNA, 27 bp, synthetic construct
  misc_feature 1..27: note = PRIMER-3
  source 1..27: mol_type = other DNA
tttctcgagatggctgaagacgaagac

SEQ ID NO: 14 - DNA, 28 bp, synthetic construct
  misc_feature 1..28: note = PRIMER-4
  source 1..28: mol_type = other DNA
tttggatcctcaattctctccataaaac

SEQ ID NO: 15 - DNA, 25 bp, synthetic construct
  misc_feature 1..25: note = PRIMER-5
  source 1..25: mol_type = other DNA
tcccatccctactcatgtggcagtg

SEQ ID NO: 16 - DNA, 34 bp, synthetic construct
  misc_feature 1..34: note = PRIMER-6
  source 1..34: mol_type = other DNA
tacaggttttcctcgagtcaaacccgacagccaa

SEQ ID NO: 17 - DNA, 40 bp, synthetic construct
  misc_feature 1..40: note = PRIMER-7
  source 1..40: mol_type = other DNA
acatcaccaagatatcatggaattatacaacggtgagagg

SEQ ID NO: 18 - DNA, 25 bp, synthetic construct
  misc_feature 1..25: note = PRIMER-8
  source 1..25: mol_type = other DNA
cactgccacatgagtagggatggga

SEQ ID NO: 19 - DNA, 40 bp, synthetic construct; identical to SEQ ID NO: 17
  misc_feature 1..40: note = PRIMER-9
  source 1..40: mol_type = other DNA

SEQ ID NO: 20 - DNA, 34 bp, synthetic construct; identical to SEQ ID NO: 16
  misc_feature 1..34: note = PRIMER-10
  source 1..34: mol_type = other DNA

SEQ ID NO: 21 - DNA, 46 bp, synthetic construct
  misc_feature 1..46: note = PRIMER-11
  source 1..46: mol_type = other DNA
acatcaccaagatatcatgttgtctattctctcttctcttttatct

SEQ ID NO: 22 - DNA, 35 bp, synthetic construct
  misc_feature 1..35: note = PRIMER-12
  source 1..35: mol_type = other DNA
tgattggccgaggcggcctcaaacccgacagccaa

SEQ ID NO: 23 - DNA, 40 bp, synthetic construct; identical to SEQ ID NO: 17
  misc_feature 1..40: note = PRIMER-13
  source 1..40: mol_type = other DNA

SEQ ID NO: 24 - DNA, 34 bp, synthetic construct; identical to SEQ ID NO: 16
  misc_feature 1..34: note = PRIMER-14
  source 1..34: mol_type = other DNA